European Patent Specification EP 3 394 262 B1, published August 28, 2024. Title: ANTISENSE ANTIBACTERIAL COMPOUNDS AND METHODS. Applicant: Geller, Bruce L. Greenberg, David. The sequence listing filed with the application follows.

SEQUENCE LISTING (35 sequences)

SEQ ID NO: 1 - DNA, 11 bp, Pseudomonas aeruginosa
  misc_feature (2)..(2): n may be thymidine or uracil
  misc_feature (5)..(5): n may be thymidine or uracil
  misc_feature (9)..(10): n may be thymidine or uracil
cncanaccnng

SEQ ID NO: 2 - DNA, 11 bp, Klebsiella pneumoniae
  misc_feature (1)..(1): n may be thymidine or uracil
  misc_feature (4)..(4): n may be thymidine or uracil
  misc_feature (7)..(7): n may be thymidine or uracil
  misc_feature (10)..(10): n may be thymidine or uracil
ngcncanacnc

SEQ ID NO: 3 - DNA, 11 bp, Pseudomonas aeruginosa
  misc_feature (3)..(5): n may be thymidine or uracil
  misc_feature (8)..(9): n may be thymidine or uracil
cgnnncannaa

SEQ ID NO: 4 - DNA, 11 bp, Pseudomonas aeruginosa
  misc_feature (1)..(3): n may be thymidine or uracil
  misc_feature (5)..(5): n may be thymidine or uracil
  misc_feature (9)..(10): n may be thymidine or uracil
nnnanccanng

SEQ ID NO: 5 - DNA, 11 bp, Pseudomonas aeruginosa
  misc_feature (4)..(6): n may be thymidine or uracil
  misc_feature (11)..(11): n may be thymidine or uracil
gcannngaccn

SEQ ID NO: 6 - DNA, 11 bp, Klebsiella pneumoniae
  misc_feature (2)..(2): n may be thymidine or uracil
  misc_feature (4)..(4): n may be thymidine or uracil
  misc_feature (6)..(7): n may be thymidine or uracil
  misc_feature (9)..(9): n may be thymidine or uracil
gncnanncncc

SEQ ID NO: 7 - DNA, 11 bp, Pseudomonas aeruginosa
  misc_feature (5)..(5): n may be thymidine or uracil
  misc_feature (7)..(7): n may be thymidine or uracil
  misc_feature (9)..(9): n may be thymidine or uracil
  misc_feature (11)..(11): n may be thymidine or uracil
gacangncnan

SEQ ID NO: 8 - DNA, 11 bp, Pseudomonas aeruginosa
  misc_feature (1)..(1): n may be thymidine or uracil
  misc_feature (4)..(5): n may be thymidine or uracil
  misc_feature (7)..(7): n may be thymidine or uracil
  misc_feature (11)..(11): n may be thymidine or uracil
nggnncngcan

SEQ ID NO: 9 - DNA, 11 bp, Pseudomonas aeruginosa
  misc_feature (3)..(5): n may be thymidine or uracil
  misc_feature (7)..(7): n may be thymidine or uracil
  misc_feature (9)..(9): n may be thymidine or uracil
agnnncncncc

SEQ ID NO: 10 - DNA, 11 bp, Pseudomonas aeruginosa
  misc_feature (2)..(3): n may be thymidine or uracil
  misc_feature (10)..(10): n may be thymidine or uracil
gnncaaacana

SEQ ID NO: 11 - DNA, 11 bp, Pseudomonas aeruginosa
  misc_feature (4)..(4): n may be thymidine or uracil
  misc_feature (7)..(7): n may be thymidine or uracil
  misc_feature (9)..(9): n may be thymidine or uracil
cgcncancnaa

SEQ ID NO: 12 - DNA, 11 bp, Pseudomonas aeruginosa
  misc_feature (1)..(2): n may be thymidine or uracil
  misc_feature (5)..(5): n may be thymidine or uracil
  misc_feature (10)..(10): n may be thymidine or uracil
nnccngccana

SEQ ID NO: 13 - DNA, 11 bp, Pseudomonas aeruginosa
  misc_feature (1)..(3): n may be thymidine or uracil
  misc_feature (6)..(6): n may be thymidine or uracil
  misc_feature (9)..(9): n may be thymidine or uracil
nnngancancg

SEQ ID NO: 14 - DNA, 11 bp, Artificial Sequence
  bacterial 23S rRNA
  misc_feature (3)..(3): n may be thymidine or uracil
  misc_feature (6)..(6): n may be thymidine or uracil
  misc_feature (8)..(8): n may be thymidine or uracil
agngcncnacc

SEQ ID NO: 15 - DNA, 11 bp, Artificial Sequence
  bacterial 23S rRNA
  misc_feature (4)..(4): n may be thymidine or uracil
  misc_feature (6)..(7): n may be thymidine or uracil
  misc_feature (9)..(9): n may be thymidine or uracil
gccngnnancc

SEQ ID NO: 16 - DNA, 11 bp, Artificial Sequence
  bacterial 16S rRNA
  misc_feature (4)..(4): n may be thymidine or uracil
ccangcagcac

SEQ ID NO: 17 - DNA, 11 bp, Artificial Sequence
  bacterial 16S rRNA
  misc_feature (1)..(2): n may be thymidine or uracil
  misc_feature (7)..(7): n may be thymidine or uracil
  misc_feature (10)..(11): n may be thymidine or uracil
nngcgcncgnn

SEQ ID NO: 18 - DNA, 11 bp, Artificial Sequence
  bacterial 16S rRNA
  misc_feature (4)..(4): n may be thymidine or uracil
  misc_feature (7)..(7): n may be thymidine or uracil
ggcngcnggca

SEQ ID NO: 19 - DNA, 11 bp, Acinetobacter baumannii
  misc_feature (1)..(1): n may be thymidine or uracil
  misc_feature (4)..(4): n may be thymidine or uracil
  misc_feature (6)..(8): n may be thymidine or uracil
  misc_feature (11)..(11): n may be thymidine or uracil
ncancnnngcn

SEQ ID NO: 20 - DNA, 11 bp, Pseudomonas aeruginosa
  misc_feature (3)..(3): n may be thymidine or uracil
  misc_feature (7)..(7): n may be thymidine or uracil
agnaacnccac

SEQ ID NO: 21 - protein, 12 aa, Artificial Sequence
  (RXR)4 cell penetrating peptide
  misc_feature (2)..(2): Xaa may be 6-aminohexanoic acid
  misc_feature (5)..(5): Xaa may be 6-aminohexanoic acid
  misc_feature (8)..(8): Xaa may be 6-aminohexanoic acid
  misc_feature (11)..(11): Xaa may be 6-aminohexanoic acid
RXRRXRRXRRXR

SEQ ID NO: 22 - protein, 10 aa, Artificial Sequence
  (RFF)3R cell penetrating peptide
RFFRFFRFFR

SEQ ID NO: 23 - protein, 14 aa, Artificial Sequence
  (RXR)4XB cell penetrating peptide
  misc_feature (2)..(2): Xaa may be 6-aminohexanoic acid
  misc_feature (5)..(5): Xaa may be 6-aminohexanoic acid
  misc_feature (8)..(8): Xaa may be 6-aminohexanoic acid
  misc_feature (11)..(11): Xaa may be 6-aminohexanoic acid
  misc_feature (13)..(13): Xaa may be 6-aminohexanoic acid
  misc_feature (14)..(14): Xaa may be beta-alanine
RXRRXRRXRRXRXX

SEQ ID NO: 24 - protein, 12 aa, Artificial Sequence
  (RFF)3RXB cell penetrating peptide
  misc_feature (11)..(11): Xaa may be 6-aminohexanoic acid
  misc_feature (12)..(12): Xaa may be beta-alanine
RFFRFFRFFRXX

SEQ ID NO: 25 - protein, 12 aa, Artificial Sequence
  (RFR)4 cell penetrating peptide
RFRRFRRFRRFR

SEQ ID NO: 26 - protein, 12 aa, Artificial Sequence
  (RYR)4 cell penetrating peptide
RYRRYRRYRRYR

SEQ ID NO: 27 - protein, 12 aa, Artificial Sequence
  (RGR)4 cell penetrating peptide
RGRRGRRGRRGR

SEQ ID NO: 28 - protein, 14 aa, Artificial Sequence
  (RFR)4XB cell penetrating peptide
  misc_feature (13)..(13): Xaa may be 6-aminohexanoic acid
  misc_feature (14)..(14): Xaa may be beta-alanine
RFRRFRRFRRFRXX

SEQ ID NO: 29 - protein, 14 aa, Artificial Sequence
  (RYR)4XB cell penetrating peptide
  misc_feature (13)..(13): Xaa may be 6-aminohexanoic acid
  misc_feature (14)..(14): Xaa may be beta-alanine
RYRRYRRYRRYRXX

SEQ ID NO: 30 - protein, 14 aa, Artificial Sequence
  (RGR)4XB cell penetrating peptide
  misc_feature (13)..(13): Xaa may be 6-aminohexanoic acid
  misc_feature (14)..(14): Xaa may be beta-alanine
RGRRGRRGRRGRXX

SEQ ID NO: 31 - protein, 12 aa, Artificial Sequence
  (RFF)3RXB cell penetrating peptide
  misc_feature (11)..(11): Xaa may be 6-aminohexanoic acid
  misc_feature (12)..(12): Xaa may be beta-alanine
RFFRFFRFFRXX

SEQ ID NO: 32 - protein, 11 aa, Artificial Sequence
  (RFF)3RG cell penetrating peptide
RFFRFFRFFRG

SEQ ID NO: 33 - protein, 7 aa, Artificial Sequence
  (R)6G cell penetrating peptide
RRRRRRG

SEQ ID NO: 34 - protein, 13 aa, Artificial Sequence
  (RXR)4G cell penetrating peptide
  misc_feature (2)..(2): Xaa may be 6-aminohexanoic acid
  misc_feature (5)..(5): Xaa may be 6-aminohexanoic acid
  misc_feature (8)..(8): Xaa may be 6-aminohexanoic acid
  misc_feature (11)..(11): Xaa may be 6-aminohexanoic acid
RXRRXRRXRRXRG

SEQ ID NO: 35 - protein, 6 aa, Artificial Sequence
  R6 cell penetrating peptide
RRRRRR